European Patent Application EP 4 296 370 A2, published December 27, 2023. Title: METHOD TO DETECT REPEAT SEQUENCE MOTIFS IN NUCLEIC ACID. Applicant: QUEST DIAGNOSTICS INVESTMENTS INCORPORATED. The sequence listing filed with the application follows.

SEQUENCE LISTING (113 sequences)

SEQ ID NO: 1 - DNA, 3240 bp, Homo sapiens
  source 1..3240: mol_type = genomic DNA
aatccatgtcccttaaagggcacagggtgtctccacagggccgcccaaaatctggtgagagagggcgtagacgcctcaccttctgcctctacgggtcacaaaagcctgggtcaccctggttgccactgttcctagttcaaagtcttcttctgtctaatccttcacccctattctcgccttccactccacctcccgctcagtcagactgcgctactttgaaccggaccaaaccaaaccaaaccaaaccaaaccaaaccagaccagacaccccctcccgcggaatcccagagaggccgaactgggataaccggatgcatttgatttcccacgccactgagtgcacctctgcagaaatgggcgttctggccctcgcgaggcagtgcgacctgtcaccgcccttcagccttcccgccctccaccaagcccgcgcacgcccggcccgcgcgtctgtctttcgacccggcaccccggccggttcccagcagcgcgcatgcgcgcgctcccaggccacttgaagagagagggcggggccgaggggctgagcccgcggggggagggaacagcgttgatcacgtgacgtggtttcagtgtttacacccgcagcgggccgggggttcggcctcagtcaggcgctcagctccgtttcggtttcacttccggtggagggccgcctctgagcgggcggcgggccgacggcgagcgcgggcggcggcggtgacggaggcgccgctgccagggggcgtgcggcagcgcggcggcggcggcggcggcggcggcggcggaggcggcggcggcggcggcggcggcggcggctgggcctcgagcgcccgcagcccacctctcgggggcgggctcccggcgctagcagggctgaagagaagatggaggagctggtggtggaagtgcggggctccaatggcgctttctacaaggtacttggctctagggcaggccccatcttcgcccttccttccctcccttttcttcttggtgtcggcgggaggcaggcccggggccctcttcccgagcaccgcgcctgggtgccagggcacgctcggcgggatgttgttgggagggaaggactggacttggggcctgttggaagcccctctccgactccgagaggccctagcgcctatcgaaatgagagaccagcgaggagagggttctctttcggcgccgagccccgccggggtgagctggggatgggcgagggccggcggcaggtactagagccgggcgggaagggccgaaatcggcgctaagtgacggcgatggcttattccccctttcctaaacatcatctcccagcgggatccgggcctgtcgtgtgggtagttgtggaggagcggggggcgcttcagccgggccgcctcctgcagcgccaagagggcttcaggtctcctttggcttctcttttccggtctagcattgggacttcggagagctccactgttctgggcgagggctgtgaagaaagagtagtaagaagcggtagtcggcaccaaatcacaatggcaactgatttttagtggcttctctttgtggatttcggaggagattttagatccaaaagtttcaggaagaccctaacatggcccagcagtgcattgaagaagttgatcatcgtgaatattcgcgtccccctttttgttaaacggggtaaattcaggaatgcacatgcttcagcgtctaaaaccattagcagcgctgctacttaaaaattgtgtgtgtgtgtttaagtttccaaagacctaaatatatgccatgaaacttcaggtaattaactgagagtatattattactagggcattttttttttaactgagcgaaaatatttttgtgcccctaagaacttgaccacatttcctttgaatttgtggtgttgcagtggactgaattgttgaggctttatataggcattcatgggtttactgtgctttttaaagttacaccattgcagatcaactaacacctttcagttttaaaaggaagatttacaaatttgatgtagcagtagtgcgtttgttggtatgtaggtgctgtataaattcatctataaattctcatttccttttgaatgtctataacctctttcaataatatcccaccttactacagtattttggcaatagaaggtgcgtgtggaaggaaggctggaaaatagctattagcagtgtccaacacaattcttaaatgtattgtagaatggcttgaatgtttcagacaggacacgtttggctataggaaaataaacaattgactttattctgtgtttaccaattttatgaagacatttggagatcagtatatttcataaatgagtaaagtatgtaaactgttccatactttgagcacaaagataaagccttttgctgtaaaaggaggcaaaaggtaaccccgcgtttatgttcttaacagtctcatgaatatgaaattgtttcagttgactctgcagtcaaaattttaatttcattgattttattgatccataatttcttctggtgagtttgcgtagaatcgttcacggtcctagattagtggttttggtcactagatttctggcactaataactataatacatatacatatatatgtgtgagtaacggctaatggttaggcaagattttgattgacctgtgatataaacttagattggatgccactaaagtttgcttatcacagagggcaagtagcacattatggccttgaagtacttattgttctcttccagcaacttatgatttgctccagtgattttgcttgcacactgactggaatataagaaatgccttctatttttgctattaattccctccttttttgttttgttttgtaacgaagttgtttaacttgaaggtgaatgaagaataggttggttgccccttagttccctgaggagaaatgttaatacttgaacaagtgtgtgtcagacaaattgctgttatgtttatttaattaagtttgatttctaagaaaatctcaaatggtctgcactgatggaagaacagtttctgtaacaaaaaagcttgaaatttttatatgacttataatactgctgtgagttttaaaagtaaagcaaaagtaaactgagttgcttgtccagtgggatggacaggaaagatgtgaaataaaaaccaatgaaaaatgaactgctgtggagaagtgttacatttatggaaaaagaaataggaaccttgttcatcaaattgatagaaaagcttttaaaactaaacaaa

SEQ ID NO: 2 - DNA, 48 bp, synthetic construct
  misc_feature 1..48: note = Description of Artificial Sequence: Synthetic primer
  source 1..48: mol_type = other DNA
tgtaaaacgacggccagtgctcagctccgtttcggtttcacttccggt

SEQ ID NO: 3 - DNA, 41 bp, synthetic construct
  misc_feature 1..41: note = Description of Artificial Sequence: Synthetic primer
  source 1..41: mol_type = other DNA
caggaaacagctatgaccctcgaggcccagccgccgccgcc

SEQ ID NO: 4 - DNA, 29 bp, synthetic construct
  misc_feature 1..29: note = Description of Artificial Sequence: Synthetic primer
  source 1..29: mol_type = other DNA
caggaaacagctatgaccccgccgccgcc

SEQ ID NO: 5 - DNA, 28 bp, synthetic construct
  misc_feature 1..28: note = Description of Artificial Sequence: Synthetic primer
  source 1..28: mol_type = other DNA
caggaaacagctatgacccgccgccgcc

SEQ ID NO: 6 - DNA, 35 bp, synthetic construct
  misc_feature 1..35: note = Description of Artificial Sequence: Synthetic primer
  source 1..35: mol_type = other DNA
caggaaacagctatgaccccgccgdcgccgccgcc

SEQ ID NO: 7 - DNA, 48 bp, synthetic construct
  misc_feature 1..48: note = Description of Artificial Sequence: Synthetic primer
  source 1..48: mol_type = other DNA
caggaaacagctatgaccccgccgccgccgccgccgccgccgccgccg

SEQ ID NO: 8 - DNA, 39 bp, synthetic construct
  misc_feature 1..39: note = Description of Artificial Sequence: Synthetic primer
  source 1..39: mol_type = other DNA
caggaaacagctatgaccccgccgccgccgccgccgccg

SEQ ID NO: 9 - DNA, 47 bp, synthetic construct
  misc_feature 1..47: note = Description of Artificial Sequence: Synthetic primer
  source 1..47: mol_type = other DNA
caggaaacagctatgaccccgccgccgccgccgccgccgccgccgcc

SEQ ID NO: 10 - DNA, 38 bp, synthetic construct
  misc_feature 1..38: note = Description of Artificial Sequence: Synthetic primer
  source 1..38: mol_type = other DNA
caggaaacagctatgaccccgccgccgccgccgccgcc

SEQ ID NO: 11 - DNA, 18 bp, synthetic construct
  misc_feature 1..18: note = Description of Artificial Sequence: Synthetic primer
  source 1..18: mol_type = other DNA
caggaaacagctatgacc

SEQ ID NO: 12 - DNA, 30 bp, synthetic construct
  misc_feature 1..30: note = Description of Artificial Sequence: Synthetic primer
  source 1..30: mol_type = other DNA
gctcagctccgtttcggtttcacttccggt

SEQ ID NO: 13 - DNA, 35 bp, synthetic construct
  misc_feature 1..35: note = Description of Artificial Sequence: Synthetic primer
  source 1..35: mol_type = other DNA
agccccgcacttccactttcggtttcacttccggt

SEQ ID NO: 14 - DNA, 10 bp, synthetic construct
  misc_feature 1..10: note = Description of Artificial Sequence: Synthetic primer
  source 1..10: mol_type = other DNA
cgccgccgcc

SEQ ID NO: 15 - DNA, 13 bp, synthetic construct
  misc_feature 1..13: note = Description of Artificial Sequence: Synthetic primer
  source 1..13: mol_type = other DNA
ccgccgaccgccg

SEQ ID NO: 16 - DNA, 13 bp, synthetic construct
  misc_feature 1..13: note = Description of Artificial Sequence: Synthetic primer
  source 1..13: mol_type = other DNA
ccgccgtccgccg

SEQ ID NO: 17 - DNA, 13 bp, synthetic construct
  misc_feature 1..13: note = Description of Artificial Sequence: Synthetic primer
  source 1..13: mol_type = other DNA
ccgccggccgccg

SEQ ID NO: 18 - DNA, 13 bp, synthetic construct
  misc_feature 1..13: note = Description of Artificial Sequence: Synthetic primer
  source 1..13: mol_type = other DNA
ccgccgcccgccg

SEQ ID NO: 19 - DNA, 19 bp, synthetic construct
  misc_feature 1..19: note = Description of Artificial Sequence: Synthetic primer
  source 1..19: mol_type = other DNA
cgccgccgacgccgccgcc

SEQ ID NO: 20 - DNA, 19 bp, synthetic construct
  misc_feature 1..19: note = Description of Artificial Sequence: Synthetic primer
  source 1..19: mol_type = other DNA
cgccgccgtcgccgccgcc

SEQ ID NO: 21 - DNA, 19 bp, synthetic construct
  misc_feature 1..19: note = Description of Artificial Sequence: Synthetic primer
  source 1..19: mol_type = other DNA
cgccgccggcgccgccgcc

SEQ ID NO: 22 - DNA, 17 bp, synthetic construct
  misc_feature 1..17: note = Description of Artificial Sequence: Synthetic primer
  source 1..17: mol_type = other DNA
cgccgccgcccgccgcc

SEQ ID NO: 23 - DNA, 18 bp, synthetic construct
  misc_feature 1..18: note = Description of Artificial Sequence: Synthetic primer
  source 1..18: mol_type = other DNA
ctcgaggcccagccgccg

SEQ ID NO: 24 - DNA, 21 bp, synthetic construct
  misc_feature 1..21: note = Description of Artificial Sequence: Synthetic primer
  source 1..21: mol_type = other DNA
ctcgaggcccagccgtcgccg

SEQ ID NO: 25 - DNA, 21 bp, synthetic construct
  misc_feature 1..21: note = Description of Artificial Sequence: Synthetic primer
  source 1..21: mol_type = other DNA
ctcgaggcccagccgacgccg

SEQ ID NO: 26 - DNA, 21 bp, synthetic construct
  misc_feature 1..21: note = Description of Artificial Sequence: Synthetic primer
  source 1..21: mol_type = other DNA
ctcgaggcccagccggcgccg

SEQ ID NO: 27 - DNA, 23 bp, synthetic construct
  misc_feature 1..23: note = Description of Artificial Sequence: Synthetic primer
  source 1..23: mol_type = other DNA
caggaaacagctatgacccgccg

SEQ ID NO: 28 - DNA, 26 bp, synthetic construct
  misc_feature 1..26: note = Description of Artificial Sequence: Synthetic primer
  source 1..26: mol_type = other DNA
caggaaacagctatgacgccgccgcc

SEQ ID NO: 29 - DNA, 30 bp, synthetic construct
  misc_feature 1..30: note = Description of Artificial Sequence: Synthetic primer
  source 1..30: mol_type = other DNA
caggaaacagctatgacccgccgaccgccg

SEQ ID NO: 30 - DNA, 30 bp, synthetic construct
  misc_feature 1..30: note = Description of Artificial Sequence: Synthetic primer
  source 1..30: mol_type = other DNA
caggaaacagctatgacccgccgtccgccg

SEQ ID NO: 31 - DNA, 30 bp, synthetic construct
  misc_feature 1..30: note = Description of Artificial Sequence: Synthetic primer
  source 1..30: mol_type = other DNA
caggaaacagctatgacccgccggccgccg

SEQ ID NO: 32 - DNA, 30 bp, synthetic construct
  misc_feature 1..30: note = Description of Artificial Sequence: Synthetic primer
  source 1..30: mol_type = other DNA
caggaaacagctatgacccgccgcccgccg

SEQ ID NO: 33 - DNA, 35 bp, synthetic construct
  misc_feature 1..35: note = Description of Artificial Sequence: Synthetic primer
  source 1..35: mol_type = other DNA
caggaaacagctatgacgccgccgacgccgccgcc

SEQ ID NO: 34 - DNA, 35 bp, synthetic construct
  misc_feature 1..35: note = Description of Artificial Sequence: Synthetic primer
  source 1..35: mol_type = other DNA
caggaaacagctatgacgccgccgtcgccgccgcc

SEQ ID NO: 35 - DNA, 35 bp, synthetic construct
  misc_feature 1..35: note = Description of Artificial Sequence: Synthetic primer
  source 1..35: mol_type = other DNA
caggaaacagctatgacgccgccggcgccgccgcc

SEQ ID NO: 36 - DNA, 33 bp, synthetic construct
  misc_feature 1..33: note = Description of Artificial Sequence: Synthetic primer
  source 1..33: mol_type = other DNA
caggaaacagctatgacgccgccgcccgccgcc

SEQ ID NO: 37 - DNA, 34 bp, synthetic construct
  misc_feature 1..34: note = Description of Artificial Sequence: Synthetic primer
  source 1..34: mol_type = other DNA
caggaaacagctatgacctcgaggcccaccgccg

SEQ ID NO: 38 - DNA, 41 bp, synthetic construct
  misc_feature 1..41: note = Description of Artificial Sequence: Synthetic primer
  source 1..41: mol_type = other DNA
caggaaacagctatgacctcgaggcccagccgtcgccgccg

SEQ ID NO: 39 - DNA, 41 bp, synthetic construct
  misc_feature 1..41: note = Description of Artificial Sequence: Synthetic primer
  source 1..41: mol_type = other DNA
caggaaacagctatgacctcgaggcccagccgacgccgccg

SEQ ID NO: 40 - DNA, 41 bp, synthetic construct
  misc_feature 1..41: note = Description of Artificial Sequence: Synthetic primer
  source 1..41: mol_type = other DNA
caggaaacagctatgacctcgaggcccagccggcgccgccg

SEQ ID NO: 41 - DNA, 10 bp, synthetic construct
  misc_feature 1..10: note = Description of Artificial Sequence: Synthetic primer
  source 1..10: mol_type = other DNA
cgcggcggcg

SEQ ID NO: 42 - DNA, 13 bp, synthetic construct
  misc_feature 1..13: note = Description of Artificial Sequence: Synthetic primer
  source 1..13: mol_type = other DNA
cggcggacggcgg

SEQ ID NO: 43 - DNA, 13 bp, synthetic construct
  misc_feature 1..13: note = Description of Artificial Sequence: Synthetic primer
  source 1..13: mol_type = other DNA
cggcggtcggcgg

SEQ ID NO: 44 - DNA, 13 bp, synthetic construct
  misc_feature 1..13: note = Description of Artificial Sequence: Synthetic primer
  source 1..13: mol_type = other DNA
cggcgggcggcgg

SEQ ID NO: 45 - DNA, 13 bp, synthetic construct
  misc_feature 1..13: note = Description of Artificial Sequence: Synthetic primer
  source 1..13: mol_type = other DNA
cggcggccggcgg

SEQ ID NO: 46 - DNA, 19 bp, synthetic construct
  misc_feature 1..19: note = Description of Artificial Sequence: Synthetic primer
  source 1..19: mol_type = other DNA
ggcggcggaggcggcggcg

SEQ ID NO: 47 - DNA, 19 bp, synthetic construct
  misc_feature 1..19: note = Description of Artificial Sequence: Synthetic primer
  source 1..19: mol_type = other DNA
ggcggcggtggcggcggcg

SEQ ID NO: 48 - DNA, 19 bp, synthetic construct
  misc_feature 1..19: note = Description of Artificial Sequence: Synthetic primer
  source 1..19: mol_type = other DNA
ggcggcgggggcggcggcg

SEQ ID NO: 49 - DNA, 17 bp, synthetic construct
  misc_feature 1..17: note = Description of Artificial Sequence: Synthetic primer
  source 1..17: mol_type = other DNA
ggcggcggccggcggcg

SEQ ID NO: 50 - DNA, 18 bp, synthetic construct
  misc_feature 1..18: note = Description of Artificial Sequence: Synthetic primer
  modified_base 6: mod_base = OTHER; note = Inosine
  source 1..18: mol_type = other DNA
cgtgcngcagcgcggcgg

SEQ ID NO: 51 - DNA, 21 bp, synthetic construct
  misc_feature 1..21: note = Description of Artificial Sequence: Synthetic primer
  modified_base 6: mod_base = OTHER; note = Inosine
  source 1..21: mol_type = other DNA
cgtgcngcagcgcggtggcgg

SEQ ID NO: 52 - DNA, 21 bp, synthetic construct
  misc_feature 1..21: note = Description of Artificial Sequence: Synthetic primer
  modified_base 6: mod_base = OTHER; note = Inosine
  source 1..21: mol_type = other DNA
cgtgcngcagcgcggaggcgg

SEQ ID NO: 53 - DNA, 21 bp, synthetic construct
  misc_feature 1..21: note = Description of Artificial Sequence: Synthetic primer
  modified_base 6: mod_base = OTHER; note = Inosine
  source 1..21: mol_type = other DNA
cgtgcngcagcgcgggggcgg

SEQ ID NO: 54 - DNA, 23 bp, synthetic construct
  misc_feature 1..23: note = Description of Artificial Sequence: Synthetic primer
  source 1..23: mol_type = other DNA
caggaaacagctatgaccggcgg

SEQ ID NO: 55 - DNA, 25 bp, synthetic construct
  misc_feature 1..25: note = Description of Artificial Sequence: Synthetic primer
  source 1..25: mol_type = other DNA
caggaaacagctatgaccggcggcg

SEQ ID NO: 56 - DNA, 30 bp, synthetic construct
  misc_feature 1..30: note = Description of Artificial Sequence: Synthetic primer
  source 1..30: mol_type = other DNA
caggaaacagctatgaccggcggacggcgg

SEQ ID NO: 57 - DNA, 30 bp, synthetic construct
  misc_feature 1..30: note = Description of Artificial Sequence: Synthetic primer
  source 1..30: mol_type = other DNA
caggaaacagctatgaccggcggtcggcgg

SEQ ID NO: 58 - DNA, 30 bp, synthetic construct
  misc_feature 1..30: note = Description of Artificial Sequence: Synthetic primer
  source 1..30: mol_type = other DNA
caggaaacagctatgaccggcggccggcgg

SEQ ID NO: 59 - DNA, 30 bp, synthetic construct
  misc_feature 1..30: note = Description of Artificial Sequence: Synthetic primer
  source 1..30: mol_type = other DNA
caggaaacagctatgaccggcgggcggcgg

SEQ ID NO: 60 - DNA, 35 bp, synthetic construct
  misc_feature 1..35: note = Description of Artificial Sequence: Synthetic primer
  source 1..35: mol_type = other DNA
caggaaacagctatgacccggcggaggcggcggcg

SEQ ID NO: 61 - DNA, 35 bp, synthetic construct
  misc_feature 1..35: note = Description of Artificial Sequence: Synthetic primer
  source 1..35: mol_type = other DNA
caggaaacagctatgacccggcggtggcggcggcg

SEQ ID NO: 62 - DNA, 35 bp, synthetic construct
  misc_feature 1..35: note = Description of Artificial Sequence: Synthetic primer
  source 1..35: mol_type = other DNA
caggaaacagctatgacccggcgggggcggcggcg

SEQ ID NO: 63 - DNA, 33 bp, synthetic construct
  misc_feature 1..33: note = Description of Artificial Sequence: Synthetic primer
  source 1..33: mol_type = other DNA
caggaaacagctatgacccggcggccggcggcg

SEQ ID NO: 64 - DNA, 33 bp, synthetic construct
  misc_feature 1..33: note = Description of Artificial Sequence: Synthetic primer
  source 1..33: mol_type = other DNA
caggaaacagctatgacccggcggtcggcggcg

SEQ ID NO: 65 - DNA, 33 bp, synthetic construct
  misc_feature 1..33: note = Description of Artificial Sequence: Synthetic primer
  source 1..33: mol_type = other DNA
caggaaacagctatgacccggcgggcggcggcg

SEQ ID NO: 66 - DNA, 33 bp, synthetic construct
  misc_feature 1..33: note = Description of Artificial Sequence: Synthetic primer
  source 1..33: mol_type = other DNA
caggaaacagctatgacccggcggacggcggcg

SEQ ID NO: 67 - DNA, 42 bp, synthetic construct
  misc_feature 1..42: note = Description of Artificial Sequence: Synthetic primer
  modified_base 24: mod_base = OTHER; note = Inosine
  source 1..42: mol_type = other DNA
caggaaacagctatgacccgtgcngcagcgcggtggcggcgg

SEQ ID NO: 68 - DNA, 42 bp, synthetic construct
  misc_feature 1..42: note = Description of Artificial Sequence: Synthetic primer
  modified_base 24: mod_base = OTHER; note = Inosine
  source 1..42: mol_type = other DNA
caggaaacagctatgacccgtgcngcagcgcggaggcggcgg

SEQ ID NO: 69 - DNA, 42 bp, synthetic construct
  misc_feature 1..42: note = Description of Artificial Sequence: Synthetic primer
  modified_base 24: mod_base = OTHER; note = Inosine
  source 1..42: mol_type = other DNA
caggaaacagctatgacccgtgcngcagcgcgggggcggcgg

SEQ ID NO: 70 - DNA, 20 bp, synthetic construct
  misc_feature 1..20: note = Description of Artificial Sequence: Synthetic oligonucleotide
  source 1..20: mol_type = other DNA
taatacgactcactataggg

SEQ ID NO: 71 - DNA, 44 bp, synthetic construct
  misc_feature 1..44: note = Description of Artificial Sequence: Synthetic primer
  source 1..44: mol_type = other DNA
caggaaacagctatgaccctcgaggcccagccgccgccgccgcc

SEQ ID NO: 72 - DNA, 47 bp, synthetic construct
  misc_feature 1..47: note = Description of Artificial Sequence: Synthetic primer
  source 1..47: mol_type = other DNA
caggaaacagctatgaccctcgaggcccagccgccgccgccgccgcc

SEQ ID NO: 73 - DNA, 38 bp, synthetic construct
  misc_feature 1..38: note = Description of Artificial Sequence: Synthetic primer
  source 1..38: mol_type = other DNA
caggaaacagctatgaccctcgaggcccagccgccgcc

SEQ ID NO: 74 - DNA, 36 bp, synthetic construct
  misc_feature 1..36: note = Description of Artificial Sequence: Synthetic primer
  source 1..36: mol_type = other DNA
caggaaacagctatgaccctcgaggcccagccgccg

SEQ ID NO: 75 - DNA, 479 bp, Homo sapiens
  source 1..479: mol_type = genomic DNA
cgccgcctgtgcagccgctgccgccgccgccgccgccgccgccgccgccgccgccgccgccgccgctgccgccccggctgccgcgccgcgccgctgcctctgccccggccgcccccgccgccgctgccgccgccggcccgcagccagccaggcgggcggcccagcccgcctgagcccgcagcggctgccgccgcagcgtcgggtcgctgggtgcgcgggctaccgcggaccgagcggacccgagtgggcgaccaggcgcttgcccgcccagtgccactgccgccgcttcctcgccggagcacaggaccagacacctccagcgcccgctgctgctgccgatgcggcccggacacttttagctgggcgggagggctggagagccgggggccgccgagaaccgccagcgagctgtgccgagagccgcgccgacccgctgcgatcagggacaggcgcccgcccgccgccgccgcctggccgct

SEQ ID NO: 76 - DNA, 20 bp, synthetic construct
  misc_feature 1..20: note = Description of Artificial Sequence: Synthetic primer
  source 1..20: mol_type = other DNA
cgccgcctgtgcagccgctg

SEQ ID NO: 77 - DNA, 20 bp, synthetic construct
  misc_feature 1..20: note = Description of Artificial Sequence: Synthetic primer
  source 1..20: mol_type = other DNA
gccccggctgccgcgccgcg

SEQ ID NO: 78 - DNA, 45 bp, synthetic construct
  misc_feature 1..45: note = Description of Artificial Sequence: Synthetic primer
  misc_feature 1..45: note = This region may encompass 1 to 15 "ccg" repeating units
  source 1..45: mol_type = other DNA
ccgccgccgccgccgccgccgccgccgccgccgccgccgccgccg

SEQ ID NO: 79 - DNA, 17 bp, synthetic construct
  misc_feature 1..17: note = Description of Artificial Sequence: Synthetic primer
  source 1..17: mol_type = other DNA
ccgccgdcgccgccgcc

SEQ ID NO: 80 - DNA, 19 bp, synthetic construct
  misc_feature 1..19: note = Description of Artificial Sequence: Synthetic primer
  source 1..19: mol_type = other DNA
cgccgccgdcgccgccgcc

SEQ ID NO: 81 - DNA, 15 bp, synthetic construct
  misc_feature 1..15: note = Description of Artificial Sequence: Synthetic primer
  source 1..15: mol_type = other DNA
ccgccgdcgccgccg

SEQ ID NO: 82 - DNA, 18 bp, synthetic construct
  misc_feature 1..18: note = Description of Artificial Sequence: Synthetic primer
  source 1..18: mol_type = other DNA
cgccgccgdcgccgccgc

SEQ ID NO: 83 - DNA, 17 bp, synthetic construct
  misc_feature 1..17: note = Description of Artificial Sequence: Synthetic primer
  source 1..17: mol_type = other DNA
gcggcggdggcggcggc

SEQ ID NO: 84 - DNA, 13 bp, synthetic construct
  misc_feature 1..13: note = Description of Artificial Sequence: Synthetic primer
  modified_base 7: mod_base = OTHER; note = a, c, t or g
  source 1..13: mol_type = other DNA
ccgccgnccgccg

SEQ ID NO: 85 - DNA, 17 bp, synthetic construct
  misc_feature 1..17: note = Description of Artificial Sequence: Synthetic primer
  modified_base 9: mod_base = OTHER; note = a, c, t or g
  source 1..17: mol_type = other DNA
cgccgccgnccgccgcc

SEQ ID NO: 86 - DNA, 16 bp, synthetic construct
  misc_feature 1..16: note = Description of Artificial Sequence: Synthetic primer
  modified_base 8: mod_base = OTHER; note = a, c, t or g
  source 1..16: mol_type = other DNA
gccgccgnccgccgcc

SEQ ID NO: 87 - DNA, 16 bp, synthetic construct
  misc_feature 1..16: note = Description of Artificial Sequence: Synthetic primer
  modified_base 9: mod_base = OTHER; note = a, c, t or g
  source 1..16: mol_type = other DNA
cgccgccgnccgccgc

SEQ ID NO: 88 - DNA, 26 bp, synthetic construct
  misc_feature 1..26: note = Description of Artificial Sequence: Synthetic primer
  source 1..26: mol_type = other DNA
ccgccgdcgccgccgdcgccgccgcc

SEQ ID NO: 89 - DNA, 28 bp, synthetic construct
  misc_feature 1..28: note = Description of Artificial Sequence: Synthetic primer
  source 1..28: mol_type = other DNA
cgccgccgdcgccgccgdcgccgccgcc

SEQ ID NO: 90 - DNA, 20 bp, synthetic construct
  misc_feature 1..20: note = Description of Artificial Sequence: Synthetic primer
  modified_base 7: mod_base = OTHER; note = a, c, t or g
  modified_base 14: mod_base = OTHER; note = a, c, t or g
  source 1..20: mol_type = other DNA
ccgccgnccgccgnccgccg

SEQ ID NO: 91 - DNA, 22 bp, synthetic construct
  misc_feature 1..22: note = Description of Artificial Sequence: Synthetic primer
  modified_base 7: mod_base = OTHER; note = a, c, t or g
  modified_base 14: mod_base = OTHER; note = a, c, t or g
  source 1..22: mol_type = other DNA
ccgccgnccgccgnccgccgcc

SEQ ID NO: 92 - DNA, 24 bp, synthetic construct
  misc_feature 1..24: note = Description of Artificial Sequence: Synthetic primer
  modified_base 9: mod_base = OTHER; note = a, c, t or g
  modified_base 16: mod_base = OTHER; note = a, c, t or g
  source 1..24: mol_type = other DNA
cgccgccgnccgccgnccgccgcc

SEQ ID NO: 93 - DNA, 11 bp, synthetic construct
  misc_feature 1..11: note = Description of Artificial Sequence: Synthetic primer
  modified_base 6: mod_base = OTHER; note = a, c, t or g
  source 1..11: mol_type = other DNA
cgccgnccgcc

SEQ ID NO: 94 - skipped

SEQ ID NO: 95 - DNA, 10 bp, synthetic construct
  misc_feature 1..10: note = Description of Artificial Sequence: Synthetic primer
  source 1..10: mol_type = other DNA
cgccgccgcc

SEQ ID NO: 96 - DNA, 45 bp, synthetic construct
  misc_feature 1..45: note = Description of Artificial Sequence: Synthetic primer
  misc_feature 1..45: note = This region may encompass 1 to 15 "cgg" repeating units
  source 1..45: mol_type = other DNA
cggcggcggcggcggcggcggcggcggcggcggcggcggcggcgg

SEQ ID NO: 97 - DNA, 17 bp, synthetic construct
  misc_feature 1..17: note = Description of Artificial Sequence: Synthetic primer
  source 1..17: mol_type = other DNA
cggcggdggcggcggcg

SEQ ID NO: 98 - DNA, 19 bp, synthetic construct
  misc_feature 1..19: note = Description of Artificial Sequence: Synthetic primer
  source 1..19: mol_type = other DNA
ggcggcggdggcggcggcg

SEQ ID NO: 99 - DNA, 15 bp, synthetic construct
  misc_feature 1..15: note = Description of Artificial Sequence: Synthetic primer
  source 1..15: mol_type = other DNA
cggcggdggcggcgg

SEQ ID NO: 100 - DNA, 18 bp, synthetic construct
  misc_feature 1..18: note = Description of Artificial Sequence: Synthetic primer
  source 1..18: mol_type = other DNA
ggcggcggdggcggcggc

SEQ ID NO: 101 - DNA, 17 bp, synthetic construct
  misc_feature 1..17: note = Description of Artificial Sequence: Synthetic primer
  source 1..17: mol_type = other DNA
gcggcggdggcggcggc

SEQ ID NO: 102 - DNA, 13 bp, synthetic construct
  misc_feature 1..13: note = Description of Artificial Sequence: Synthetic primer
  modified_base 7: mod_base = OTHER; note = a, c, t or g
  source 1..13: mol_type = other DNA
cggcggncggcgg

SEQ ID NO: 103 - DNA, 17 bp, synthetic construct
  misc_feature 1..17: note = Description of Artificial Sequence: Synthetic primer
  modified_base 9: mod_base = OTHER; note = a, c, t or g
  source 1..17: mol_type = other DNA
ggcggcggncggcggcg

SEQ ID NO: 104 - DNA, 16 bp, synthetic construct
  misc_feature 1..16: note = Description of Artificial Sequence: Synthetic primer
  modified_base 8: mod_base = OTHER; note = a, c, t or g
  source 1..16: mol_type = other DNA
gcggcggncggcggcg

SEQ ID NO: 105 - DNA, 15 bp, synthetic construct
  misc_feature 1..15: note = Description of Artificial Sequence: Synthetic primer
  modified_base 8: mod_base = OTHER; note = a, c, t or g
  source 1..15: mol_type = other DNA
gcggcggncggcggc

SEQ ID NO: 106 - DNA, 26 bp, synthetic construct
  misc_feature 1..26: note = Description of Artificial Sequence: Synthetic primer
  source 1..26: mol_type = other DNA
cggcggdggcggcggdggcggcggcg

SEQ ID NO: 107 - DNA, 28 bp, synthetic construct
  misc_feature 1..28: note = Description of Artificial Sequence: Synthetic primer
  source 1..28: mol_type = other DNA
ggcggcggdggcggcggdggcggcggcg

SEQ ID NO: 108 - DNA, 20 bp, synthetic construct
  misc_feature 1..20: note = Description of Artificial Sequence: Synthetic primer
  modified_base 7: mod_base = OTHER; note = a, c, t or g
  modified_base 14: mod_base = OTHER; note = a, c, t or g
  source 1..20: mol_type = other DNA
cggcggncggcggncggcgg

SEQ ID NO: 109 - DNA, 22 bp, synthetic construct
  misc_feature 1..22: note = Description of Artificial Sequence: Synthetic primer
  modified_base 7: mod_base = OTHER; note = a, c, t or g
  modified_base 14: mod_base = OTHER; note = a, c, t or g
  source 1..22: mol_type = other DNA
cggcggncggcggncggcggcg

SEQ ID NO: 110 - DNA, 24 bp, synthetic construct
  misc_feature 1..24: note = Description of Artificial Sequence: Synthetic primer
  modified_base 9: mod_base = OTHER; note = a, c, t or g
  modified_base 16: mod_base = OTHER; note = a, c, t or g
  source 1..24: mol_type = other DNA
ggcggcggncggcggncggcggcg

SEQ ID NO: 111 - DNA, 11 bp, synthetic construct
  misc_feature 1..11: note = Description of Artificial Sequence: Synthetic primer
  modified_base 6: mod_base = OTHER; note = a, c, t or g
  source 1..11: mol_type = other DNA
ggcggncggcg

SEQ ID NO: 112 - skipped

SEQ ID NO: 113 - DNA, 10 bp, synthetic construct
  misc_feature 1..10: note = Description of Artificial Sequence: Synthetic primer
  source 1..10: mol_type = other DNA
ggcggcggcg